European Patent Specification EP 3 283 630 B1, published July 26, 2023. Title: OLIGONUCLEOTIDE FRAGMENT, AND METHOD AS WELL AS APPLICATION OF SELECTIVE AMPLIFICTION OF VARIANT OF TARGET NUCLEIC ACID SEQUENCE USING THE SAME. Applicant: Nuhigh Biotechnologies Co. Ltd. The sequence listing filed with the application follows.

SEQUENCE LISTING (20 sequences)

SEQ ID NO: 1 - DNA, 302 bp, artificial sequence
  misc_feature
tttccagcatggtgagggctgaggtgacccttgtctctgtgttcttgtcccccccagcttgtggagcctcttacacccagtggagaagctcccaaccaagctctcttgaggatcttgaaggaaactgaattcaaaaagatcaaagtgctgagctccggtgcgttcggcacggtgtataaggtaaggtccctggcacaggcctctgggctgggccgcagggcctctcatggtctggtggggagcccagagtccttgcaagctgtatatttccatcatctactttactctttgtttcactgagt

SEQ ID NO: 2 - DNA, 302 bp, artificial sequence
  misc_feature
tttccagcatggtgagggctgaggtgacccttgtctctgtgttcttgtcccccccagcttgtggagcctcttacacccagtggagaagctcccaaccaagctctcttgaggatcttgaaggaaactgaattcaaaaagatcaaagtgctgggctccggtgcgttcggcacggtgtataaggtaaggtccctggcacaggcctctgggctgggccgcagggcctctcatggtctggtggggagcccagagtccttgcaagctgtatatttccatcatctactttactctttgtttcactgagt

SEQ ID NO: 3 - DNA, 19 bp, artificial sequence
  misc_feature
tatacaccgtgccgaacgc

SEQ ID NO: 4a - DNA, 5 bp, artificial sequence
  misc_feature
ctggg

SEQ ID NO: 4b - DNA, 16 bp, artificial sequence
  misc_feature
caccgtgccgaacgca

SEQ ID NO: 5 - DNA, 283 bp, artificial sequence
  misc_feature
ctggccaccatgcgaagccacactgacgtgcctctccctccctccaggaagcctacgtgatggccagcgtggacaacccccacgtgtgccgcctgctgggcatctgcctcacctccaccgtgcagctcatcatgcagctcatgcccttcggctgcctcctggactatgtccgggaacacaaagacaatattggctcccagtacctgctcaactggtgtgtgcagatcgcaaaggtaatcagggaagggagatacggggaggggagataaggagccaggatcct

SEQ ID NO: 6 - DNA, 283 bp, artificial sequence
  misc_feature
ctggccaccatgcgaagccacactgacgtgcctctccctccctccaggaagcctacgtgatggccagcgtggacaacccccacgtgtgccgcctgctgggcatctgcctcacctccaccgtgcagctcatcacgcagctcatgcccttcggctgcctcctggactatgtccgggaacacaaagacaatattggctcccagtacctgctcaactggtgtgtgcagatcgcaaaggtaatcagggaagggagatacggggaggggagataaggagccaggatcct

SEQ ID NO: 7 - DNA, 17 bp, artificial sequence
  misc_feature
aggcagccgaagggcat

SEQ ID NO: 8a - DNA, 10 bp, artificial sequence
  misc_feature
gcgtgatgag

SEQ ID NO: 8b - DNA, 18 bp, artificial sequence
  misc_feature
cctcacctccaccgtgca

SEQ ID NO: 9 - DNA, 14 bp, artificial sequence
  misc_feature
gtgctgagctccgg

SEQ ID NO: 10 - DNA, 21 bp, artificial sequence
  misc_feature
tggagcctcttacacccagtg

SEQ ID NO: 11a - DNA, 7 bp, artificial sequence
  misc_feature
gcccagc

SEQ ID NO: 11b - DNA, 26 bp, artificial sequence
  misc_feature
ggaaactgaattcaaaaagatcaaag

SEQ ID NO: 12 - DNA, 306 bp, artificial sequence
  misc_feature
ttcggggtgcatcgctggtaacatccacccagatcactgggcagcatgtggcaccatctcacaattgccagttaacgtcttccttctctctctgtcatagggactctggatcccagaaggtgagaaagttaaaattcccgtcgctatcaagacatctccgaaagccaacaaggaaatcctcgatgtgagtttctgctttgctgtgtgggggtccatggctctgaacctcaggcccaccttttctcatgtctggcagctgctctgctctagaccctgctcatctccacatcctaaatgttcactttc

SEQ ID NO: 13 - DNA, 321 bp, artificial sequence
  misc_feature
ttcggggtgcatcgctggtaacatccacccagatcactgggcagcatgtggcaccatctcacaattgccagttaacgtcttccttctctctctgtcatagggactctggatcccagaaggtgagaaagttaaaattcccgtcgctatcaaggaattaagagaagcaacatctccgaaagccaacaaggaaatcctcgatgtgagtttctgctttgctgtgtgggggtccatggctctgaacctcaggcccaccttttctcatgtctggcagctgctctgctctagaccctgctcatctccacatcctaaatgttcactttc

SEQ ID NO: 14 - DNA, 20 bp, artificial sequence
  misc_feature
ttccttgttggctttcggag

SEQ ID NO: 15 - DNA, 37 bp, artificial sequence
  misc_feature
cttctcttaattcgttaaaattcccgtcgctatcaag

SEQ ID NO: 16a - DNA, 7 bp, artificial sequence
  misc_feature
gcccagc

SEQ ID NO: 16b - DNA, 26 bp, artificial sequence
  misc_feature
ggaaactgaattcaaaaagatcaaag